European Patent Application EP 4 613 330 A1, published September 10, 2025. Title: MRNA VACCINE ENCODING FUSION ANTIGEN AGAINST MPOX AND SEVERE ACUTE RESPIRATORY SYNDROME CORONAVIRUS 2. Applicant: ACADEMY OF MILITARY MEDICAL SCIENCE, ACADEMY OF MILITARY  SCIENCE, PEOPLE'S LIBERATION ARMY OF CHINA. The sequence listing filed with the application follows.

SEQUENCE LISTING (15 sequences)

SEQ ID NO: 1 - DNA, 1212 bp, synthetic construct
  source 1..1212: mol_type = other DNA
atggacgccatgaagagaggcctgtgctgtgtgctgctgctgtgcggcgccgtgttcgtgtccaacagcatgggcgccgccgccagcatccagaccacagtgaataccctgagcgagaggatcagctccaagctggagcaggaggccaatgccagcgcccagaccaagtgtgatatcgagatcggcaatttctacatcaggcagaaccacggctgtaacatcacagtgaagaacatgtgctccgccgatgccgatgcccagctggacgccgtgctgtccgccgctaccgagacctacagcggcctgacacctgagcagaaggcctacgtgcctgccatgttcaccgccgccctgaacatccagacctccgtgaataccgtggtgagggatttcgagaattacgtgaagcagacatgcaacagcagcgccgtggtggataacaagctgaagatccagaatgtgatcatcgacgagtgctacggcgcccccggcagccctacaaacctggagtttatcaacacaggcagcagcaagggcaactgtgccatcaaggccctgatgcagctgacaaccaaggccacaacaacaaacctgtgcccctttcacgaggtgttcaacgccacaaccttcgcctccgtgtacgcctggaataggaagaggatctccaactgcgtggccgactactccgtgatctacaacttcgccccctttttcgcctttaagtgttacggcgtgagccctacaaagctgaatgacctgtgtttcaccaatgtgtacgccgattcctttgtgatcagaggcaacgaggtgtcccagatcgcccccggccagacaggcaatatcgccgactacaactacaagctgcctgatgacttcaccggctgtgtgatcgcctggaatagcaacaagctggattccaaggtgggcggcaactacaactacctgtacaggctgttcagaaagagcaagctgaagccttttgagagagacatctccaccgagatctaccaggccggcaacagaccctgtaatggcgtggagggcttcaattgctactcccccctgcagtcctacggcttcaggcccacatacggcgtgggccaccagccctacagagtggtggtgctgagctttgagctgctgcacgcccctgccaccgtgtgcggaccaaagaagtccacaaatctggtgaagaacaagtgcgtgaacttt

SEQ ID NO: 2 - protein, 404 aa, synthetic construct
MDAMKRGLCCVLLLCGAVFVSNSMGAAASIQTTVNTLSERISSKLEQEANASAQTKCDIEIGNFYIRQNHGCNITVKNMCSADADAQLDAVLSAATETYSGLTPEQKAYVPAMFTAALNIQTSVNTVVRDFENYVKQTCNSSAVVDNKLKIQNVIIDECYGAPGSPTNLEFINTGSSKGNCAIKALMQLTTKATTTNLCPFHEVFNATTFASVYAWNRKRISNCVADYSVIYNFAPFFAFKCYGVSPTKLNDLCFTNVYADSFVIRGNEVSQIAPGQTGNIADYNYKLPDDFTGCVIAWNSNKLDSKVGGNYNYLYRLFRKSKLKPFERDISTEIYQAGNRPCNGVEGFNCYSPLQSYGFRPTYGVGHQPYRVVVLSFELLHAPATVCGPKKSTNLVKNKCVNF

SEQ ID NO: 3 - DNA, 2091 bp, synthetic construct
  source 1..2091: mol_type = other DNA
atggatgccatgaagagaggcctgtgctgcgtgctgctgctgtgtggcgccgtgtttgtgagcaatagcatgggcgccgccgccagcatccagaccaccgttaataccctgagcgagagaatctccagcaagctggagcaggaggccaatgccagcgcccagaccaagtgtgatatcgagatcggcaacttctacatcaggcagaaccacggctgtaatatcaccgtgaagaacatgtgttccgccgacgccgacgcccagctggacgctgttctgagcgccgccaccgagacctactccggcctgacacccgagcagaaggcctacgtgcccgccatgttcacagccgccctgaacatccagacaagcgtgaacacagtggtgagagatttcgagaattacgtgaagcagacatgcaactcctccgccgtggtggataacaagctgaagatccagaatgtgatcatcgatgagtgctacggcgcccctggctcccccacaaacctggagtttatcaataccggctcctccaagggcaattgcgccatcaaggccctgatgcagctgaccacaaaggccaccaccacaaatctgtgccccttccacgaggtgttcaacgccaccacattcgcctccgtgtacgcctggaataggaagagaatctccaactgcgtggccgattacagcgtgatctacaatttcgccccctttttcgcctttaagtgctacggcgtgagccccaccaagctgaatgacctgtgctttaccaatgtgtacgccgatagctttgtgatcaggggcaatgaggtgagccagatcgcccctggccagaccggcaatatcgccgattacaactacaagctgcccgacgatttcacaggctgtgtgatcgcctggaatagcaataagctggattccaaggtgggcggcaactacaattacctgtacaggctgttcagaaagtccaagctgaagcccttcgagagagacatcagcaccgagatctaccaggccggcaacagaccttgcaatggcgtggagggcttcaactgctacagccctctgcagagctacggcttcaggcccacctacggcgtgggccaccagccatacagggtggtggtgctgtccttcgagctgctgcacgcccctgccacagtgtgcggccctaagaagtccaccaacctggtgaagaataagtgcgtgaattttagagtgcagcctaccgagagcatcgtgaggtttcccaacatcacaaatctgtgtcccttccacgaagtgtttaatgccaccacatttgcctccgtgtatgcctggaacagaaagagaatcagcaactgtgtggccgactacagcgtgatctataactttgcccccttcttcgcctttaaatgttacggcgtgtcccctaccaagctgaacgatctgtgttttaccaatgtctacgccgattccttcgtgatcagaggcaacgaggtgtcccagatcgccccaggccagacaggcaatatcgctgactacaactacaaactgcccgatgattttaccggctgtgtgattgcctggaatagtaacaagctggacagcaagccctccggcaactacaactacctgtaccggctgctgagaaagtccaaactgaagccctttgagagagacatttccacagagatctaccaagccggcaacaagccctgtaagggcgtggccggccctaattgctactcccctctgcagtcctacggctttagacccacatacggcgtgggacaccagccctacagggtggtcgtgctgtcctttgagctgctgcatgcccccgccacagtgtgtggcaaggagagctgcaacggcctgtactaccagggcagctgttacatcctgcacagcgactacaagtccttcgaggacgccaaggccaattgcgccgccgagagctccacactgcctaacaagtccgacgtgctgacaacatggctgatcgattacgtggaggatacctggggctccgatggcaatcctatcaccaagacaacatccgactaccaggattccgatgtgtcccaggaggtgagaaagtacttctgcacc

SEQ ID NO: 4 - protein, 697 aa, synthetic construct
MDAMKRGLCCVLLLCGAVFVSNSMGAAASIQTTVNTLSERISSKLEQEANASAQTKCDIEIGNFYIRQNHGCNITVKNMCSADADAQLDAVLSAATETYSGLTPEQKAYVPAMFTAALNIQTSVNTVVRDFENYVKQTCNSSAVVDNKLKIQNVIIDECYGAPGSPTNLEFINTGSSKGNCAIKALMQLTTKATTTNLCPFHEVFNATTFASVYAWNRKRISNCVADYSVIYNFAPFFAFKCYGVSPTKLNDLCFTNVYADSFVIRGNEVSQIAPGQTGNIADYNYKLPDDFTGCVIAWNSNKLDSKVGGNYNYLYRLFRKSKLKPFERDISTEIYQAGNRPCNGVEGFNCYSPLQSYGFRPTYGVGHQPYRVVVLSFELLHAPATVCGPKKSTNLVKNKCVNFRVQPTESIVRFPNITNLCPFHEVFNATTFASVYAWNRKRISNCVADYSVIYNFAPFFAFKCYGVSPTKLNDLCFTNVYADSFVIRGNEVSQIAPGQTGNIADYNYKLPDDFTGCVIAWNSNKLDSKPSGNYNYLYRLLRKSKLKPFERDISTEIYQAGNKPCKGVAGPNCYSPLQSYGFRPTYGVGHQPYRVVVLSFELLHAPATVCGKESCNGLYYQGSCYILHSDYKSFEDAKANCAAESSTLPNKSDVLTTWLIDYVEDTWGSDGNPITKTTSDYQDSDVSQEVRKYFCT

SEQ ID NO: 5 - DNA, 19 bp, synthetic construct
  source 1..19: mol_type = other DNA
taatacgactcactatagg

SEQ ID NO: 6 - DNA, 41 bp, synthetic construct
  source 1..41: mol_type = other DNA
gggactcttctggtccccacagactcagagagaacgccacc

SEQ ID NO: 7 - DNA, 110 bp, synthetic construct
  source 1..110: mol_type = other DNA
gctggagcctcggtggcctagcttcttgccccttgggcctccccccagcccctcctccccttcctgcacccgtacccccgtggtctttgaataaagtctgagtgggcggc

SEQ ID NO: 8 - DNA, 585 bp, synthetic construct
  source 1..585: mol_type = other DNA
atggacgccatgaagagaggcctgtgctgtgtgctgctgctgtgtggcgccgtgttcgtgtccaactccatgggcgccgccgccagcatccagacaaccgtgaacaccctgtccgagagaatcagcagcaagctggagcaggaggccaatgcctccgcccagacaaagtgcgacatcgagatcggcaacttttacatcaggcagaaccacggctgcaacatcaccgtgaagaatatgtgcagcgccgatgccgatgcccagctggatgccgtgctgagcgccgctaccgagacctactccggcctgacccctgagcagaaggcctacgtgcccgccatgttcaccgccgccctgaacatccagaccagcgtgaacaccgtggtgagagattttgagaactacgtgaagcagacatgcaactccagcgccgtggtggacaataagctgaagatccagaacgtgatcatcgatgagtgctacggcgcccctggctcccctacaaacctggagtttatcaacaccggctccagcaagggcaactgtgccatcaaggccctgatgcagctgaccaccaaggccaccaca

SEQ ID NO: 9 - DNA, 696 bp, synthetic construct
  source 1..696: mol_type = other DNA
atggacgccatgaagaggggcctgtgctgtgtgctgctgctgtgcggcgccgtgttcgtgagcaattccacaaacctgtgtccttttcacgaggtgttcaacgccacaaccttcgccagcgtgtacgcctggaacaggaagagaatcagcaattgtgtggccgactacagcgtgatctacaacttcgcccctttctttgcctttaagtgctacggcgtgagccctacaaagctgaacgacctgtgctttacaaatgtgtacgccgatagcttcgtgatcagaggcaacgaggtgagccagatcgcccctggccagaccggcaacatcgccgattacaattacaagctgcccgacgattttaccggctgtgtgatcgcctggaacagcaacaagctggactccaaggtgggcggcaattacaattacctgtacaggctgtttaggaagtccaagctgaagccttttgagagggatatctccaccgagatctaccaggccggcaacaggccctgtaacggcgtggagggcttcaattgctacagccctctgcagtcctacggcttcagacctacctacggcgtgggccaccagccttacagggtggtggtgctgagcttcgagctgctgcacgcccccgccacagtgtgcggacctaagaagtccacaaatctggtgaagaataagtgtgtgaacttc

SEQ ID NO: 10 - DNA, 324 bp, synthetic construct
  source 1..324: mol_type = other DNA
atggacgccatgaagaggggcctgtgttgtgtgctgctgctgtgcggcgccgtgttcgtgtccaacagcaaggagagctgtaatggcctgtactaccagggcagctgttacatcctgcacagcgactacaagtccttcgaggacgccaaggccaattgtgccgccgagagcagcacactgcctaataagagcgacgtgctgacaacctggctgatcgattacgtggaggatacctggggcagcgacggcaatcctatcacaaagacaacctccgactaccaggattccgatgtgtcccaggaggtgaggaagtacttttgcaca

SEQ ID NO: 11 - RNA, 855 nt, synthetic construct
  source 1..855: mol_type = other RNA
gggactcttctggtccccacagactcagagagaacgccaccatggacgccatgaagagaggcctgtgctgtgtgctgctgctgtgtggcgccgtgttcgtgtccaactccatgggcgccgccgccagcatccagacaaccgtgaacaccctgtccgagagaatcagcagcaagctggagcaggaggccaatgcctccgcccagacaaagtgcgacatcgagatcggcaacttttacatcaggcagaaccacggctgcaacatcaccgtgaagaatatgtgcagcgccgatgccgatgcccagctggatgccgtgctgagcgccgctaccgagacctactccggcctgacccctgagcagaaggcctacgtgcccgccatgttcaccgccgccctgaacatccagaccagcgtgaacaccgtggtgagagattttgagaactacgtgaagcagacatgcaactccagcgccgtggtggacaataagctgaagatccagaacgtgatcatcgatgagtgctacggcgcccctggctcccctacaaacctggagtttatcaacaccggctccagcaagggcaactgtgccatcaaggccctgatgcagctgaccaccaaggccaccacatgataataggctggagcctcggtggcctagcttcttgccccttgggcctccccccagcccctcctccccttcctgcacccgtacccccgtggtctttgaataaagtctgagtgggcggcaaaaaaaaaaaaaaaaaaaaaaaaaaaaaaaaaaaaaaaaaaaaaaaaaaaaaaaaaaaaaaaaaaaaaaaaaaaaaaaaaaaaaaaaaaaaaaaaaaaaaaaaaaaaaa

SEQ ID NO: 12 - RNA, 966 nt, synthetic construct
  source 1..966: mol_type = other RNA
gggactcttctggtccccacagactcagagagaacgccaccatggacgccatgaagaggggcctgtgctgtgtgctgctgctgtgcggcgccgtgttcgtgagcaattccacaaacctgtgtccttttcacgaggtgttcaacgccacaaccttcgccagcgtgtacgcctggaacaggaagagaatcagcaattgtgtggccgactacagcgtgatctacaacttcgcccctttctttgcctttaagtgctacggcgtgagccctacaaagctgaacgacctgtgctttacaaatgtgtacgccgatagcttcgtgatcagaggcaacgaggtgagccagatcgcccctggccagaccggcaacatcgccgattacaattacaagctgcccgacgattttaccggctgtgtgatcgcctggaacagcaacaagctggactccaaggtgggcggcaattacaattacctgtacaggctgtttaggaagtccaagctgaagccttttgagagggatatctccaccgagatctaccaggccggcaacaggccctgtaacggcgtggagggcttcaattgctacagccctctgcagtcctacggcttcagacctacctacggcgtgggccaccagccttacagggtggtggtgctgagcttcgagctgctgcacgcccccgccacagtgtgcggacctaagaagtccacaaatctggtgaagaataagtgtgtgaacttctgataataggctggagcctcggtggcctagcttcttgccccttgggcctccccccagcccctcctccccttcctgcacccgtacccccgtggtctttgaataaagtctgagtgggcggcaaaaaaaaaaaaaaaaaaaaaaaaaaaaaaaaaaaaaaaaaaaaaaaaaaaaaaaaaaaaaaaaaaaaaaaaaaaaaaaaaaaaaaaaaaaaaaaaaaaaaaaaaaaaaa

SEQ ID NO: 13 - RNA, 594 nt, synthetic construct
  source 1..594: mol_type = other RNA
gggactcttctggtccccacagactcagagagaacgccaccatggacgccatgaagaggggcctgtgttgtgtgctgctgctgtgcggcgccgtgttcgtgtccaacagcaaggagagctgtaatggcctgtactaccagggcagctgttacatcctgcacagcgactacaagtccttcgaggacgccaaggccaattgtgccgccgagagcagcacactgcctaataagagcgacgtgctgacaacctggctgatcgattacgtggaggatacctggggcagcgacggcaatcctatcacaaagacaacctccgactaccaggattccgatgtgtcccaggaggtgaggaagtacttttgcacatgataataggctggagcctcggtggcctagcttcttgccccttgggcctccccccagcccctcctccccttcctgcacccgtacccccgtggtctttgaataaagtctgagtgggcggcaaaaaaaaaaaaaaaaaaaaaaaaaaaaaaaaaaaaaaaaaaaaaaaaaaaaaaaaaaaaaaaaaaaaaaaaaaaaaaaaaaaaaaaaaaaaaaaaaaaaaaaaaaaaaa

SEQ ID NO: 14 - RNA, 1482 nt, synthetic construct
  source 1..1482: mol_type = other RNA
gggactcttctggtccccacagactcagagagaacgccaccatggacgccatgaagagaggcctgtgctgtgtgctgctgctgtgcggcgccgtgttcgtgtccaacagcatgggcgccgccgccagcatccagaccacagtgaataccctgagcgagaggatcagctccaagctggagcaggaggccaatgccagcgcccagaccaagtgtgatatcgagatcggcaatttctacatcaggcagaaccacggctgtaacatcacagtgaagaacatgtgctccgccgatgccgatgcccagctggacgccgtgctgtccgccgctaccgagacctacagcggcctgacacctgagcagaaggcctacgtgcctgccatgttcaccgccgccctgaacatccagacctccgtgaataccgtggtgagggatttcgagaattacgtgaagcagacatgcaacagcagcgccgtggtggataacaagctgaagatccagaatgtgatcatcgacgagtgctacggcgcccccggcagccctacaaacctggagtttatcaacacaggcagcagcaagggcaactgtgccatcaaggccctgatgcagctgacaaccaaggccacaacaacaaacctgtgcccctttcacgaggtgttcaacgccacaaccttcgcctccgtgtacgcctggaataggaagaggatctccaactgcgtggccgactactccgtgatctacaacttcgccccctttttcgcctttaagtgttacggcgtgagccctacaaagctgaatgacctgtgtttcaccaatgtgtacgccgattcctttgtgatcagaggcaacgaggtgtcccagatcgcccccggccagacaggcaatatcgccgactacaactacaagctgcctgatgacttcaccggctgtgtgatcgcctggaatagcaacaagctggattccaaggtgggcggcaactacaactacctgtacaggctgttcagaaagagcaagctgaagccttttgagagagacatctccaccgagatctaccaggccggcaacagaccctgtaatggcgtggagggcttcaattgctactcccccctgcagtcctacggcttcaggcccacatacggcgtgggccaccagccctacagagtggtggtgctgagctttgagctgctgcacgcccctgccaccgtgtgcggaccaaagaagtccacaaatctggtgaagaacaagtgcgtgaacttttgataataggctggagcctcggtggcctagcttcttgccccttgggcctccccccagcccctcctccccttcctgcacccgtacccccgtggtctttgaataaagtctgagtgggcggcaaaaaaaaaaaaaaaaaaaaaaaaaaaaaaaaaaaaaaaaaaaaaaaaaaaaaaaaaaaaaaaaaaaaaaaaaaaaaaaaaaaaaaaaaaaaaaaaaaaaaaaaaaaaaa

SEQ ID NO: 15 - RNA, 2361 nt, synthetic construct
  source 1..2361: mol_type = other RNA
gggactcttctggtccccacagactcagagagaacgccaccatggatgccatgaagagaggcctgtgctgcgtgctgctgctgtgtggcgccgtgtttgtgagcaatagcatgggcgccgccgccagcatccagaccaccgttaataccctgagcgagagaatctccagcaagctggagcaggaggccaatgccagcgcccagaccaagtgtgatatcgagatcggcaacttctacatcaggcagaaccacggctgtaatatcaccgtgaagaacatgtgttccgccgacgccgacgcccagctggacgctgttctgagcgccgccaccgagacctactccggcctgacacccgagcagaaggcctacgtgcccgccatgttcacagccgccctgaacatccagacaagcgtgaacacagtggtgagagatttcgagaattacgtgaagcagacatgcaactcctccgccgtggtggataacaagctgaagatccagaatgtgatcatcgatgagtgctacggcgcccctggctcccccacaaacctggagtttatcaataccggctcctccaagggcaattgcgccatcaaggccctgatgcagctgaccacaaaggccaccaccacaaatctgtgccccttccacgaggtgttcaacgccaccacattcgcctccgtgtacgcctggaataggaagagaatctccaactgcgtggccgattacagcgtgatctacaatttcgccccctttttcgcctttaagtgctacggcgtgagccccaccaagctgaatgacctgtgctttaccaatgtgtacgccgatagctttgtgatcaggggcaatgaggtgagccagatcgcccctggccagaccggcaatatcgccgattacaactacaagctgcccgacgatttcacaggctgtgtgatcgcctggaatagcaataagctggattccaaggtgggcggcaactacaattacctgtacaggctgttcagaaagtccaagctgaagcccttcgagagagacatcagcaccgagatctaccaggccggcaacagaccttgcaatggcgtggagggcttcaactgctacagccctctgcagagctacggcttcaggcccacctacggcgtgggccaccagccatacagggtggtggtgctgtccttcgagctgctgcacgcccctgccacagtgtgcggccctaagaagtccaccaacctggtgaagaataagtgcgtgaattttagagtgcagcctaccgagagcatcgtgaggtttcccaacatcacaaatctgtgtcccttccacgaagtgtttaatgccaccacatttgcctccgtgtatgcctggaacagaaagagaatcagcaactgtgtggccgactacagcgtgatctataactttgcccccttcttcgcctttaaatgttacggcgtgtcccctaccaagctgaacgatctgtgttttaccaatgtctacgccgattccttcgtgatcagaggcaacgaggtgtcccagatcgccccaggccagacaggcaatatcgctgactacaactacaaactgcccgatgattttaccggctgtgtgattgcctggaatagtaacaagctggacagcaagccctccggcaactacaactacctgtaccggctgctgagaaagtccaaactgaagccctttgagagagacatttccacagagatctaccaagccggcaacaagccctgtaagggcgtggccggccctaattgctactcccctctgcagtcctacggctttagacccacatacggcgtgggacaccagccctacagggtggtcgtgctgtcctttgagctgctgcatgcccccgccacagtgtgtggcaaggagagctgcaacggcctgtactaccagggcagctgttacatcctgcacagcgactacaagtccttcgaggacgccaaggccaattgcgccgccgagagctccacactgcctaacaagtccgacgtgctgacaacatggctgatcgattacgtggaggatacctggggctccgatggcaatcctatcaccaagacaacatccgactaccaggattccgatgtgtcccaggaggtgagaaagtacttctgcacctgataataggctggagcctcggtggcctagcttcttgccccttgggcctccccccagcccctcctccccttcctgcacccgtacccccgtggtctttgaataaagtctgagtgggcggcaaaaaaaaaaaaaaaaaaaaaaaaaaaaaaaaaaaaaaaaaaaaaaaaaaaaaaaaaaaaaaaaaaaaaaaaaaaaaaaaaaaaaaaaaaaaaaaaaaaaaaaaaaaaaa